European Patent Application EP 4 603 106 A1, published August 20, 2025. Title: POPULATIONS OF SMALL EXTRACELLULAR VESICLES FOR USE IN THE TREATMENT OR PREVENTION OF ISCHEMIA. Applicant: UNIVERSIDADE DE SANTIAGO DE COMPOSTELA. The sequence listing filed with the application follows.

SEQUENCE LISTING (9 sequences)

SEQ ID NO: 1 - protein, 552 aa, synthetic construct
MAEKQKHDGRVKIGHYVLGDTLGVGTFGKVKIGEHQLTGHKVAVKILNRQKIRSLDVVGKIKREIQNLKLFRHPHIIKLYQVISTPTDFFMVMEYVSGGELFDYICKHGRVEEVEARRLFQQILSAVDYCHRHMVVHRDLKPENVLLDAQMNAKIADFGLSNMMSDGEFLRTSCGSPNYAAPEVISGRLYAGPEVDIWSCGVILYALLCGTLPFDDEHVPTLFKKIRGGVFYIPDYLNRSVATLLMHMLQVDPLKRATIKDIREHEWFKQDLPSYLFPEDPSYDANVIDDEAVKEVCEKFECTESEVMNSLYSGDPQDQLAVAYHLIIDNRRIMNQASEFYLASSPPSGSFMDDSAMHIPPGLKPHPERMPPLIADSPKARCPLDALNTTKPKSLAVKKAKWHLGIRSQSKACDIMAEVYRAMKQLGFEWKVVNAYHLRVRRKNPVTGNYVKMSLQLYLVDSRSYLLDFKSIDDEVVEQRSGSSTPQRSCSAAGLHRARSSFDSSTAENHSLSGSLTGSLTGSTLSSASPRLGSHTMDFFEMCASLITALAR

SEQ ID NO: 2 - protein, 563 aa, synthetic construct
MEQKLISEEDLGGGEKQKHDGRVKIGHYVLGDTLGVGTFGKVKIGEHQLTGHKVAVKILNRQKIRSLDVVGKIKREIQNLKLFRHPHIIKLYQVISTPTDFFMVMEYVSGGELFDYICKHGRVEEVEARRLFQQILSAVDYCHRHMVVHRDLKPENVLLDAQMNAKIAAFGLSNMMSDGEFLRTSCGSPNYAPEVISGRLYAGPEVDIWSCGVILYALLCGTLPFDDEHVPTLFKKIRGGVFYIPEYLNRSIATLLMHMLQVDPLKRATIKDIREHEWFKQDLPSYLFPEDPSYDANVIDDEAVKEVCEKFECTESEVMNSLYSGDPQDQLAVAYHLIIDNRRIMNQASEFYLASSPPTGSFMDDSAMHIPPGLKPHPERMPPLIADSPKARCPLDALNTTKPKSLAVKKAKWHLGIRSQSKPYDIMAEVYRAMKQLDFEWKVVNAYHLRVRRKNPVTGNYVKMSLQLYLVDNRSYLLDFKSIDDEVVEQRSGSSTPQRSCSAAGLHRPRSSVDSSTAENHSLSGSLTGSLTGSTLSSASPRLGSHTMDFFEMCASLITALAR

SEQ ID NO: 3 - DNA, 1667 bp, synthetic construct
  source 1..1667: mol_type = other DNA
ggcgagaagcagaagcacgacgggcgtgtgaagatcggacactacgtgctgggggacaccctgggcgtcggcaccttcggcaaagtgaagattggagaacatcaattgacaggccataaagtggcagttaagatcttaaatagacagaagattcgcagtttagatgttgttggaaaaataaaacgagaaattcaaaatcttaaactctttcgtcatcctcatattatcaaactctaccaagtgatcagcactccaacagacttttttatggtaatggaatatgtgtctggaggtgaattgttcgactacatctgtaaacacgggagggttgaagaggtggaagctcgccggctcttccagcagattctgtctgccgtggactactgtcacaggcacatggttgtccacagggacctgaagccagagaacgtgttgctggacgcccagatgaatgctaagatagctgccttcggactctctaatatgatgtcagatggtgaatttctacgaactagctgtggatcgccaaattatgcagcaccggaggtcatctcaggaaggctgtatgcgggtcctgaggttgatatctggagctgtggtgttatcctgtatgcccttctctgtggcaccctcccgttcgacgatgagcacgtgcctacgctctttaagaagatccgagggggtgtgttctacatcccggagtatctcaaccgttctattgccactctgctgatgcacatgctgcaggtggaccccttgaagcgagcaactatcaaagacatacgagagcatgaatggttcaagcaagatttgcccagttacctctttcctgaagacccctcctatgatgctaacgtcattgatgatgaggctgtgaaagaagtatgtgaaaaatttgagtgtacagaatcagaagtgatgaacagtttatacagtggtgaccctcaagaccagctcgcagtggcttatcatctcatcattgacaatcggagaataatgaaccaagccagtgagttctacctcgcctccagtcctccaacgggttccttcatggacgatagtgccatgcatattccccccggcctgaaaccacatcctgaaaggatgccacctctcatagcagacagccccaaagcacgctgtccactggatgcactcaacacaactaagcccaaatctttagctgtgaaaaaagccaagtggcaccttgggatccgaagccagagcaaaccatacgacattatggcggaggtgtaccgagctatgaagcagctggactttgaatggaaggtagtgaatgcataccatcttcgagtaagaagaaaaaacccagtgactggcaattacgtgaaaatgagcttacagctttacctggttgacaatcggagctatcttctagactttaaaagcatcgatgatgaggtggtggagcagaggtctggttcttcaacacctcagcgctcctgttctgctgccggcctccacagacctcggtcaagtgtcgattccagcacagccgagaaccattcactgtctggctctctcactggttctttgactggcagcactttgtcctccgcttccccgcgcctgggcagtcataccatggatttttttgaaatgtgcgccagtcttatcactgctttagcccgttgataataactcac

SEQ ID NO: 4 - DNA, 500 bp, synthetic construct
  source 1..500: mol_type = other DNA
tacggtaaatggcccgcctggctgaccgcccaacgacccccgcccattgacgtcaataatgacgtatgttcccatagtaacgccaatagggactttccattgacgtcaatgggtggagtatttacggtaaactgcccacttggcagtacatcaagtgtatcatatgccaagtacgccccctattgacgtcaatgacggtaaatggcccgcctggcattatgcccagtacatgaccttatgggactttcctacttggcagtacatctacgtattagtcatcgctattaccatggtgatgcggttttggcagtacatcaatgggcgtggatagcggtttgactcacggggatttccaagtctccaccccattgacgtcaatgggagtttgttttggcaccaaaatcaacgggactttccaaaatgtcgtaacaactccgccccattgacgcaaatgggcggtaggcgtgtacggtgggaggtctatataagcagagctcgtt

SEQ ID NO: 5 - protein, 449 aa, synthetic construct
MCLSPVKGAKLILIFLFLGAVQSNALIVNLTDSKGTCLYARYTIWMPENPRPGTPCDIFTNSRGKRASNGSGGAEWEMNFTITYETTNQTNKTITIAVPDKATHDGSSCGDDRNSAKIMIQFGFAVSWAVNFTKEASHYSIHDIVLSYNTSDSTVFPGAVAKGVHTVKNPENFKVPLDVIFKCNSVLTYNLTPVVQKYWGIHLQAFVQNGTVSKNEQVCEEDQTPTTVAPIIHTTAPSTTTTLTPTSTPTPTPTPTPTVGNYSIRNGNTTCLLATMGLQLNITEEKVPFIFNINPATTNFTGSCQPQSAQLRLNNSQIKYLDFIFAVKNEKRFYLKEVNVYMYLANGSAFNISNKNLSFWDAPLGSSYMCNKEQVLSVSRAFQINTFNLKVQPFNVTKGQYSTAQECSLDDDTILIPIIVGAGLSGLIIVIVIAYLIGRRKTYAGYQTL

SEQ ID NO: 6 - DNA, 7905 bp, synthetic construct
  source 1..7905: mol_type = other DNA
ttaagctagcatcatcaataatataccttattttggattgaagccaatatgataatgagggggtggagtttgtgacgtggcgcggggcgtgggaacggggcgggtgacgtagtagtgtggcggaagtgtgatgttgcaagtgtggcggaacacatgtaagcgacggatgtggcaaaagtgacgtttttggtgtgcgccggtgtacacaggaagtgacaattttcgcgcggttttaggcggatgttgtagtaaatttgggcgtaaccgagtaagatttggccattttcgcgggaaaactgaataagaggaagtgaaatctgaataattttgtgttactcatagcgcgtaatatttgtctagggagatcagcctgcaggtcgttacataacttacggtaaatggcccgcctggctgaccgcccaacgacccccgcccattgacgtcaataatgacgtatgttcccatagtaacgccaatagggactttccattgacgtcaatgggtggagtatttacggtaaactgcccacttggcagtacatcaagtgtatcatatgccaagtacgccccctattgacgtcaatgacggtaaatggcccgcctggcattatgcccagtacatgaccttatgggactttcctacttggcagtacatctacgtattagtcatcgctattaccatggtgatgcggttttggcagtacatcaatgggcgtggatagcggtttgactcacggggatttccaagtctccaccccattgacgtcaatgggagtttgttttggcaccaaaatcaacgggactttccaaaatgtcgtaacaactccgccccattgacgcaaatgggcggtaggcgtgtacggtgggaggtctatataagcagagctcgtttagtgaaccgtcagatggtaccgtttaaactcgaggtcgacggtatcgataagcttgatatcgaattcgccatggagcagaagcttatctccgaggaggacctcggtggcggcgagaagcagaagcacgacgggcgtgtgaagatcggacactacgtgctgggggacaccctgggcgtcggcaccttcggcaaagtgaagattggagaacatcaattgacaggccataaagtggcagttaagatcttaaatagacagaagattcgcagtttagatgttgttggaaaaataaaacgagaaattcaaaatcttaaactctttcgtcatcctcatattatcaaactctaccaagtgatcagcactccaacagacttttttatggtaatggaatatgtgtctggaggtgaattgttcgactacatctgtaaacacgggagggttgaagaggtggaagctcgccggctcttccagcagattctgtctgccgtggactactgtcacaggcacatggttgtccacagggacctgaagccagagaacgtgttgctggacgcccagatgaatgctaagatagctgccttcggactctctaatatgatgtcagatggtgaatttctacgaactagctgtggatcgccaaattatgcagcaccggaggtcatctcaggaaggctgtatgcgggtcctgaggttgatatctggagctgtggtgttatcctgtatgcccttctctgtggcaccctcccgttcgacgatgagcacgtgcctacgctctttaagaagatccgagggggtgtgttctacatcccggagtatctcaaccgttctattgccactctgctgatgcacatgctgcaggtggaccccttgaagcgagcaactatcaaagacatacgagagcatgaatggttcaagcaagatttgcccagttacctctttcctgaagacccctcctatgatgctaacgtcattgatgatgaggctgtgaaagaagtatgtgaaaaatttgagtgtacagaatcagaagtgatgaacagtttatacagtggtgaccctcaagaccagctcgcagtggcttatcatctcatcattgacaatcggagaataatgaaccaagccagtgagttctacctcgcctccagtcctccaacgggttccttcatggacgatagtgccatgcatattccccccggcctgaaaccacatcctgaaaggatgccacctctcatagcagacagccccaaagcacgctgtccactggatgcactcaacacaactaagcccaaatctttagctgtgaaaaaagccaagtggcaccttgggatccgaagccagagcaaaccatacgacattatggcggaggtgtaccgagctatgaagcagctggactttgaatggaaggtagtgaatgcataccatcttcgagtaagaagaaaaaacccagtgactggcaattacgtgaaaatgagcttacagctttacctggttgacaatcggagctatcttctagactttaaaagcatcgatgatgaggtggtggagcagaggtctggttcttcaacacctcagcgctcctgttctgctgccggcctccacagacctcggtcaagtgtcgattccagcacagccgagaaccattcactgtctggctctctcactggttctttgactggcagcactttgtcctccgcttccccgcgcctgggcagtcataccatggatttttttgaaatgtgcgccagtcttatcactgctttagcccgttgataataactcaccaccggctagagcggccgccacagcggggagatccagacatgataagatacattgatgagtttggacaaaccacaactagaatgcagtgaaaaaaatgctttatttgtgaaatttgtgatgctattgctttatttgtaaccattataagctgcaataaacaagttaacaacaacaattgcattcattttatgtttcaggttcagggggaggtgtgggaggttttttaaagcaagtaaaacctctacaaatgtggtatggctgattatgatccggctgcctcgcgcgtttcggtgatgacggtgaaaacctctgacacatgcagctcccggagacggtcacagcttgtctgtaagcggatgccgggagcagacaagcccgtcagggcgcgtcagcgggtgttggcgggtgtcggggcgcagccatgaggtcgactctagtccccgcggtggcagatctggaaggtgctgaggtacgatgagacccgcaccaggtgcagaccctgcgagtgtggcggtaaacatattaggaaccagcctgtgatgctggatgtgaccgaggagctgaggcccgatcacttggtgctggcctgcacccgcgctgagtttggctctagcgatgaagatacagattgaggtactgaaatgtgtgggcgtggcttaagggtgggaaagaatatataaggtgggggtcttatgtagttttgtatctgttttgcagcagccgccgccgccatgagcaccaactcgtttgatggaagcattgtgagctcatatttgacaacgcgcatgcccccatgggccggggtgcgtcagaatgtgatgggctccagcattgatggtcgccccgtcctgcccgcaaactctactaccttgacctacgagaccgtgtctggaacgccgttggagactgcagcctccgccgccgcttcagccgctgcagccaccgcccgcgggattgtgactgactttgctttcctgagcccgcttgcaagcagtgcagcttcccgttcatccgcccgcgatgacaagttgacggctcttttggcacaattggattctttgacccgggaacttaatgtcgtttctcagcagctgttggatctgcgccagcaggtttctgccctgaaggcttcctcccctcccaatgcggtttaaaacataaataaaaaaccagactctgtttggatttggatcaagcaagtgtcttgctgtctttatttaggggttttgcgcgcgcggtaggcccgggaccagcggtctcggtcgttgagggtcctgtgtattttttccaggacgtggtaaaggtgactctggatgttcagatacatgggcataagcccgtctctggggtggaggtagcaccactgcagagcttcatgctgcggggtggtgttgtagatgatccagtcgtagcaggagcgctgggcgtggtgcctaaaaatgtctttcagtagcaagctgattgccaggggcaggcccttggtgtaagtgtttacaaagcggttaagctgggatgggtgcatacgtggggatatgagatgcatcttggactgtatttttaggttggctatgttcccagccatatccctccggggattcatgttgtgcagaaccaccagcacagtgtatccggtgcacttgggaaatttgtcatgtagcttagaaggaaatgcgtggaagaacttggagacgcccttgtgacctccaagattttccatgcattcgtccataatgatggcaatgggcccacgggcggcggcctgggcgaagatatttctgggatcactaacgtcatagttgtgttccaggatgagatcgtcataggccatttttacaaagcgcgggcggagggtgccagactgcggtataatggttccatccggcccaggggcgtagttaccctcacagatttgcatttcccacgctttgagttcagatggggggatcatgtctacctgcggggcgatgaagaaaacggtttccggggtaggggagatcagctgggaagaaagcaggttcctgagcagctgcgacttaccgcagccggtgggcccgtaaatcacacctattaccgggtgcaactggtagttaagagagctgcagctgccgtcatccctgagcaggggggccacttcgttaagcatgtccctgactcgcatgttttccctgaccaaatccgccagaaggcgctcgccgcccagcgatagcagttcttgcaaggaagcaaagtttttcaacggtttgagaccgtccgccgtaggcatgcttttgagcgtttgaccaagcagttccaggcggtcccacagctcggtcacctgctctacggcatctcgatccagcatatctcctcgtttcgcgggttggggcggctttcgctgtacggcagtagtcggtgctcgtccagacgggccagggtcatgtctttccacgggcgcagggtcctcgtcagcgtagtctgggtcacggtgaaggggtgcgctccgggctgcgcgctggccagggtgcgcttgaggctggtcctgctggtgctgaagcgctgccggtcttcgccctgcgcgtcggccaggtagcatttgaccatggtgtcatagtccagcccctccgcggcgtggcccttggcgcgcagcttgcccttggaggaggcgccgcacgaggggcagtgcagacttttgagggcgtagagcttgggcgcgagaaataccgattccggggagtaggcatccgcgccgcaggccccgcagacggtctcgcattccacgagccaggtgagctctggccgttcggggtcaaaaaccaggtttcccccatgctttttgatgcgtttcttacctctggtttccatgagccggtgtccacgctcggtgacgaaaaggctgtccgtgtccccgtatacagacttgagaggcctgtcctcgaccgatgcccttgagagccttcaacccagtcagctccttccggtgggcgcggggcatgactatcgtcgccgcacttatgactgtcttctttatcatgcaactcgtaggacaggtgccggcagcgctctgggtcattttcggcgaggaccgctttcgctggagcgcgacgatgatcggcctgtcgcttgcggtattcggaatcttgcacgccctcgctcaagccttcgtcactggtcccgccaccaaacgtttcggcgagaagcaggccattatcgccggcatggcggccgacgcgctgggctacgtcttgctggcgttcgcgacgcgaggctggatggccttccccattatgattcttctcgcttccggcggcatcgggatgcccgcgttgcaggccatgctgtccaggcaggtagatgacgaccatcagggacagcttcaaggccagcaaaaggccaggaaccgtaaaaaggccgcgttgctggcgtttttccataggctccgcccccctgacgagcatcacaaaaatcgacgctcaagtcagaggtggcgaaacccgacaggactataaagataccaggcgtttccccctggaagctccctcgtgcgctctcctgttccgaccctgccgcttaccggatacctgtccgcctttctcccttcgggaagcgtggcgctttctcatagctcacgctgtaggtatctcagttcggtgtaggtcgttcgctccaagctgggctgtgtgcacgaaccccccgttcagcccgaccgctgcgccttatccggtaactatcgtcttgagtccaacccggtaagacacgacttatcgccactggcagcagccactggtaacaggattagcagagcgaggtatgtaggcggtgctacagagttcttgaagtggtggcctaactacggctacactagaaggacagtatttggtatctgcgctctgctgaagccagttaccttcggaaaaagagttggtagctcttgatccggcaaacaaaccaccgctggtagcggtggtttttttgtttgcaagcagcagattacgcgcagaaaaaaaggatctcaagaagatcctttgatcttttctacggggtctgacgctcagtggaacgaaaactcacgttaagggattttggtcatgagattatcaaaaaggatcttcacctagatccttttaaattaaaaatgaagttttaaatcaatctaaagtatatatgagtaaacttggtctgacagttaccaatgcttaatcagtgaggcacctatctcagcgatctgtctatttcgttcatccatagttgcctgactccccgtcgtgtagataactacgatacgggagggcttaccatctggccccagtgctgcaatgataccgcgagacccacgctcaccggctccagatttatcagcaataaaccagccagccggaagggccgagcgcagaagtggtcctgcaactttatccgcctccatccagtctattaattgttgccgggaagctagagtaagtagttcgccagttaatagtttgcgcaacgttgttgccattgctgcaggcatcgtggtgtcacgctcgtcgtttggtatggcttcattcagctccggttcccaacgatcaaggcgagttacatgatcccccatgttgtgcaaaaaagcggttagctccttcggtcctccgatcgttgtcagaagtaagttggccgcagtgttatcactcatggttatggcagcactgcataattctcttactgtcatgccatccgtaagatgcttttctgtgactggtgagtactcaaccaagtcattctgagaatagtgtatgcggcgaccgagttgctcttgcccggcgtcaacacgggataataccgcgccacatagcagaactttaaaagtgctcatcattggaaaacgttcttcggggcgaaaactctcaaggatcttaccgctgttgagatccagttcgatgtaacccactcgtgcacccaactgatcttcagcatcttttactttcaccagcgtttctgggtgagcaaaaacaggaaggcaaaatgccgcaaaaaagggaataagggcgacacggaaatgttgaatactcatactcttcctttttcaatattattgaagcatttatcagggttattgtctcatgagcggatacatatttgaatgtatttagaaaaataaacaaataggggttccgcgcacatttccccgaaaagtgccacctgacgtctaagaaaccattattatcatgacattaacctataaaaataggcgtatcacgaggccctttcgtcttcaagaaaattaa

SEQ ID NO: 7 - protein, 14 aa, synthetic construct
ACGTGNNNNACGTG

SEQ ID NO: 8 - DNA, 8201 bp, synthetic construct
  source 1..8201: mol_type = other DNA
gggtaggcggcggcggcggcggtggcggcggtagcggcggcggcagcggtagcggcggcggcgctcagagcccgcggcagggggagcccgtgcgccgaacatggctgagaagcagaagcacgacgggcgggtgaagatcggacactacgtcctgggggacaccctgggcgtcggcaccttcggcaaagtgaagattggagaacaccaattgacaggccataaagtggcagttaagatcttaaatagacagaagattcgcagtttagatgttgttggaaaaataaaacgagaaattcaaaatcttaaactctttcgtcatcctcatattatcaaactctaccaggtgatcagcactccgacagacttttttatggtaatggaatatgtgtctggaggtgaattgttcgactacatctgcaaacatgggcgggttgaagaggtggaagcgcgccggctcttccagcagatcctgtctgccgtggattactgtcacaggcatatggttgtccatagggacctgaagccagagaatgtgctgctggatgcccagatgaacgctaagatagctgactttggactatctaatatgatgtcagatggtgaatttctacgaactagctgtggatcgccaaattatgcagcacctgaggtcatctcaggaaggctgtatgcaggtcccgaggtcgatatctggagctgtggtgtcatcctgtatgcccttctctgtggcaccctccctttcgatgatgagcacgtgcctacgctcttcaagaagatccgagggggtgtgttttacatcccagactatctcaaccgttctgtcgccactctgctgatgcacatgctccaggtggaccccctgaagcgagcgactatcaaagacatacgagaacatgaatggtttaaacaggatttgcccagctacctatttcctgaagacccctcctacgatgcgaatgtcattgacgatgaggctgtgaaggaagtctgtgagaaattcgagtgtacagagtcagaagtgatgaatagtctgtatagtggtgaccctcaagaccagcttgcagtggcttatcatcttatcattgacaatcggagaataatgaaccaagccagtgagttctacctcgcctctagtcctccatcaggttcttttatggatgacagcgccatgcatattcctccaggcttgaaaccacatccagaaaggatgccgcctctcatcgcagacagccccaaagcacgctgtccactggatgcactcaacacaacgaagcccaagtctctagctgtgaaaaaagccaagtggcatcttggaatccgaagccagagcaaagcgtgtgacattatggctgaagtgtaccgagctatgaagcagctgggttttgaatggaaggtagtgaatgcataccatcttcgagtaagaagaaaaaacccagtgactggcaactatgtgaaaatgagcttacagctttacctggtagacagtcggagctatcttctggacttcaaaagcatcgatgatgaggtggtggagcagaggtctggttcttcaacaccccagcgctcctgttctgctgcgggcctccacagagcacggtcaagttttgattccagcacagctgagaaccactccctttctggctctctcactggctctttgactggcagcactttgtcctcggcatccccgcgcctgggcagtcacaccatggatttttttgaaatgtgcgccagtcttatcactgctttagctcgttgattatccacccctggtctctgtctttctgtcacccccctgtgaaatcacatacactctttaaattattatctcactcggtattacgtgctctgcaatagaagttggtgtgaacattcccaggtgacatgcagtgttattgaaatcaccgaaaacacagaaatccagcattctgtttactcgtagaactctgtaactctcctgtgcctgtgacaagtttgcatgggtagtactgggtgagtgtggtggcgcttgctaacttacacctgtgaattcgctgtagatggcaagcacacctcactgatgaacgaacccgctgaggtaggggtggttcaatgggcctccttccttcatgtttcctgtacgtaaatccggtttacctcctaaacttcagcagctgttaggctgcctgggcactcttgcacaagaagattaagatatagaataactgttagggaaatattatttcaatgtagaaatctgaaaatcctgtccccctaaatattagaaaccaaagtcttttaaattatttctgcaaatactgcctagtattagccattaagactgtgtttctgataacaggagcctaatctcccagcttcctgacagttgtgcaaggcgcctagttaaatcacaccaccaccaagcaaaacaaaaccatgcaaaattagtacacagttcaatgagacaagcaaaataccaacaacagtctcttaaaagaaaattctactctatgatcttgtttgtgtttatcagactggggtagctgggaggagggccggcagtcatggccctctggcatgtttgctaattcccttaacatttgttatcgatgccacctcctccctccgtcttcctcaggagcctctgtcttgctcaatgcttttccctttcattaatcctttagctaaaaaccttgctttggccatcatgtctttgtatacttccaaagcttgatctctgtgaccttcactgttgaacctgattggacagggaagccttaaatatttaaaagtatattctcctggaatacgtatatgtgttgtttacatatatatacatatgtattgacacatcagtgcttttaatcaaaaaaaaaccaaacatttttgtgcaagttttttttttaatttaagacaaaaaagcactatattgcaagatagattaagttaattgattatatgttgttttggtaaaagtattttaaattatgtgtaatttatctaataattatttattcatctattgtatttatgttgtaattttaaaaatcattgatctgattcaccctagaaaatattaagctcttgaaaaaaaaaaaaagcaacattgccttgacaggtttctcttcaccaaaaattgtatattttctatttaccaagaagcaaatgagactgttagaccaggtttctcatgagattccagaagacaagtttgtctgtctttaaatagctttttgaatcaggaatttgcatcatatcacatcagataactttgtagttcttttaaaaagatggtcaatatttatcactccaacttctcaatggtaaaataaaagaatctttgcccactgattgagaaggagagtgtataatttaaggtaccttaagtttaatctttgaaagattgccatcttgtggcaatagatggtaattttagtagttattttaataccaatacttagtcctgcctgggttatctaatgtgttttatgaatgtggcatagttctgacttctccaaatgtgtctgtatccttgtttgtggggtgggggagagatcaccttatgatgtttgcctaatcatggcatggaaggccttgaagtaaggaactgaatagattctttacctctaataacagcatccacaacagtgatgaaggcaggaaggaggcagaatgcttttagtctagtgaatttaaaccaaaattactttatatgaatgattatgatgctattcaagagctaaaagttatttactattgtcttaattcattccagtattatgaatacccaggttgacagttacctgctgaatttcaggagaactgaaggtcattttgtttcttttaacattttaagacataattatttaatgaatctagatgatagagtaagttggttttcagagagaattcagtgactcatctcgaaaagcagaggcaggaattcagtcacagcatagggatttgttgctcttggaaacagagaaggaaagaattctttgcaaatttacagttcctacatttcagtcaatcctatgggtatggtaggtactgagtttagagcagcctatcctcttggatcgtgcggagaataactattaagttatagatgtggtatgtcttggaaacggagtccatctgtttccaaaatagtatttcctaaaacaaagaaatcccacaaaataattttgaaatacattgtgttctgctctgcaccttgcagaggacagtgactattaactcgaaagacttgcagactttgagaaaaaaacaaaacaaaaagaccccacataactgcaaaaaccctactttgcccaaactagtttactcttttaaaacgtttgctgagtctggttgcttacctgtaatacgactggggagtatgaggcaggaagatacgttggggcctaagaactagatagatagcaagaccttgtttcaaattgaaacaataaaggaactgtagcatcccataagaacataggagaaacgattgtctctgagcgccacggtgtggtcgttagtgacagtgagtaacacctcttccccagagcctgatgctaattcagatctgctccattgaccatgcacatagggtcatcctgagtctgggcttgtaccacatgctggttttcctaatcatatgatgctttttaggtagaacatctattctttttttcccttagagggtgactgaaaagtcctagacaaggttacttatggaaaaccagaagagtaagagagcagtggctttctgttgtggcttcatggatagcaagccagttttattcatttttcaatggccactgaacgttttctaagtccttttatttaggaaaccaaaattgaagctatctcaaagtaaatctacagggagagagaaaaccaaaccattcacaagttagggttctgttttgatcaagaactcttgtaaaaggcccttgcaacatctggttatctgcagagagaagctaggagcctaagctaagcagaaacattaagaccctctgtgttagggaattgggtatatgtagcacagtaattctctactttatgcaagtaagtattcaagaatatttacttaattctcaatctactcttttcttagctagtttgtactcagggaacacaaatttaatacaaatgaaatgaaacacaatttggaaaataatcgtaaacaaccgaatcagatttttatactgcttcatctgtagtctctgctaacatgcaagcatgcttagttaatgtgggccccacactgatgttcataagacttaacagcctggaacatacctaacacagataccacagctctgcctggtcactcccagggtgaagtctcatacctaaatgtgagactgcccgtagacttgtctgctttgtgtttggttcagtctggcaacttgtccttcagttctctgtggcttgttaagtagggcttatggcttagtagttcttggcaactctgttgaaaactctggatagtaagtgtgatctaggacttggcctcaatttaaaaccctaaaatgaaagggatggacacagagctatcgtccctctgagctctgaagtcatgccttgtttactacttcagagcgtcagtgtgagtgttcacattttatgtatttgtttgctagtatgagtgttttttccttagtccgaggcatttcaaaggtacactaaccaaaagtacttggactactggaatgcaaaactgaaaacatggtgtggatttagcattcattagaagatgactgctaggtagcagtggtggggcccatgcatttccaggtctgctagtgctccctcgcagtacccagtccagtaagcaggctcactgcagttgatcatcttctgggctgaacagaaagagtttgtgaaacatctgagagtcaagtaataaaaataaacactggtgtgttgtttgtaagtcctggaatgacatatagtagttataagtgaatgtagttagtctaattataaaagctagttgattgcactaactagatgtaattttgtgaaatatttatgattatattgattttattataagtatttataagttattgagggtgcttaaaatccagaaaaatctctaggacatatttttttttctgaaattgtatttatatgatttgggtgtagggagttttatactggtgactgagcccaggcttcccgtgtaagaagcaagggcttaacttcaacctcaatcccctggccctctacatgattctgaaagtccaggcgctctttgtcgaggaaaattagccccagcccgatctaaatgatcacagtttgtgactgctagctgaactaggcttatctaaatttcattttggccatttttaattttgtgcataaatgagatgacactgtttttatacagtgtgtctctctgagctacctaatcactattggctctgatagaagttcaccaagcctttttaaacttggaaacgtaacttaagttaatgagctttaagtcatgcatatatgtatgtgtatatatacatatggattatgtaaacaagttagcagcggcgtctttatcagcggcgcctttccttgaatatttatgatgcggttgatgctactgaacagtaataccgtgaggaacaggccccagtctagactctagactggatggagttttgattaagcttcttcagccataacctgttcagaatcaggtccaatccagacgttatcagactgcaggcctgtattttgtgagccaacattaatgtttactgccagccttgcatagcagtgccggttgcgactgcatgtgacttttagtaactgtagtttatgtctaaaagcagttcaagttttatagaggtaattcatgattatttgaacaagcagggtgggtaattcaaatatatttaaagtgcaattaaggaaattctagggtataatattctttccagttttaaaaaaaatagttaaggatttttagaatgtcctagaatgaaaaaaattttttttggacagactttttaaaaaacaaggtttatacagatttttttttttaattcaaggtttgctactttgtgtttatttaaatttgcaaagagaaaccgaagcctcctaggaaagagttgcattgttatttttctcctgctagtctgaatgtgcattttcacagctaaaagtcacttgtaaataaggtttgttaccacattcgaagcccatgttttctaaatggagaacattttcccagaatcaaagagacatagacccactgtctacacaaagaaagaaagcgtacctggtgccttctcaaataattgtagagtcaaagtgaacgtgttccaagtctgccccaccccaccccctctcctgttcctcgggttctctgtgacctacctgtccctcccacagacggtcacaggatttgcttctgccctttcagttctacttgaccaaacctcacagcatcaccagtgacgttcttcactgaatacattttctctttcacttatttcactttttaaagccacctgggaaaatatttggctgccttcttatgcttttaaaatgaatgcaattattagcagtgtttatatttgaaagtttataaaggaaagaaattcagagctaaggactgactcttaattggatctaattccctgtgtgttacgatagcagcacaagttatgtaaccttgtgtagttttctcttgtacaaaatgtggatgataacctacctcacagatgtgtgtgagaagccgtttcaaagcccctaagtaggggtttatagtcccatcctcagtgtcaatcctcccttttttactagacacctttgagaatggtaggatgagtatcttgtttttagatgtcatatgtaataagggcatagtgctgagaatgtttaagacacagtttcacaaatcatagtgttcttactgtaagacacttaaaaatttcttgaaaacctcaaatgtttaaatatcgaatctgtcttttgtttcaataaatattgttattcaaagtgttgtctgaagctgccttaatgtaccaaaatacaactgtcaaaactgttcacaactatattcatggttgtactgttttgagtgttcattttgaagttgctatgaactatgaccttgaaggatagtattttgatattattttggtaggaatagttgtggttttttttttcatcatgtttaacagtgacttttgtgtgtaaaaaataaaactgaaacttggcag

SEQ ID NO: 9 - DNA, 453 bp, synthetic construct
  source 1..453: mol_type = other DNA
ctagaatcccaaaacaaactggttattgtggtaggtcatttgtttggcagaaagaaaactcgagaaatttctctggccgttattcgttattctctcttttctttttgggtctctccctctctgcactaatgctctctcactctgtcacacagtaaacggcatactgctctcgttggttcgagagagcgcgcctcgaatgttcgcgaaaagagcgccggagtataaatagaggcgcttcgtctacggagcgacaattcaattcaaacaagcaaagtgaacacgtcgctaagcgaaagctaagcaaataaacaagcgcagctgaacaagctaaacaatctgcagtaaagtgcaagttaaagtgaatcaattaaaagtaaccagcaaccaagtaaatcaactgcaactactgaaatctgccaagaagtaattattgaatacaagaagagaactctg